European Patent Specification EP 3 296 390 B1, published January 4, 2023. Title: Method for Preparing Stem Cell Clone Suitable for Inducing Differentiation into Somatic Cells. Applicant: KYOTO UNIVERSITY Megakaryon Corporation. The sequence listing filed with the application follows.

SEQUENCE LISTING (6 sequences)

SEQ ID NO: 1 - protein, 20 aa, Artificial
  A synthesized caspase inhibitor peptide.
  MOD_RES (1)..(1): ACETYLATION
  MOD_RES (20)..(20): Acetaldehyde-modified aspartic acid.
AAVALLPAVLLALLAPYVAD

SEQ ID NO: 2 - protein, 20 aa, Artificial
  A synthesized caspase inhibitor peptide.
  MOD_RES (1)..(1): ACETYLATION
  MOD_RES (20)..(20): Acetaldehyde-modified aspartic acid.
AAVALLPAVLLALLAPDEVD

SEQ ID NO: 3 - protein, 20 aa, Artificial
  A synthesized caspase inhibitor peptide.
  MOD_RES (1)..(1): ACETYLATION
  MOD_RES (20)..(20): Acetaldehyde-modified aspartic acid.
AAVALLPAVLLALLAPLEVD

SEQ ID NO: 4 - protein, 20 aa, Artificial
  A synthesized caspase inhibitor peptide.
  MOD_RES (1)..(1): ACETYLATION
  MOD_RES (20)..(20): Acetaldehyde-modified aspartic acid.
AAVALLPAVLLALLAPIETD

SEQ ID NO: 5 - protein, 20 aa, Artificial
  A synthesized caspase inhibitor peptide.
  MOD_RES (1)..(1): ACETYLATION
  MOD_RES (20)..(20): Acetaldehyde-modified aspartic acid.
AAVALLPAVLLALLAPLEHD

SEQ ID NO: 6 - protein, 4 aa, Artificial
  A synthesized caspase inhibitor peptide.
  MOD_RES (1)..(1): Benzyloxycarbonyl-modified aspartic acid.
  MOD_RES (4)..(4): Fluoromethylketone-modified aspartic acid.
DEVD